European Patent Application EP 4 209 134 A1, published July 12, 2023. Title: METHOD OF PREPARING FERMENTED FOOD BY USING NOVEL RHIZOPUS MICROSPORUS STRAIN, AND FERMENTED FOOD. Applicant: Industrial Technology Research Institute. The sequence listing filed with the application follows.

SEQUENCE LISTING (3 sequences)

SEQ ID NO: 1 - DNA, 660 bp, Rhizopus microsporus
  source 1..660: mol_type = genomic DNA
cattaactaatgtattggcactttactgggatttacttctcagtattgtttgcttctatactgtgaacctctggcgatgaaggtcgtaactgaccttcgggagagactcaggacatataggctataatgggtaggcctgttctggggtttgatcgatgccaatcaggattacctttcttcctttgggaaggaaggtgcctggtaccctttaccatataccatgaattcagaattgaaagtataatataataacaacttttaacaatggatctcttggttctcgcatcgatgaagaacgtagcaaagtgcgataactagtgtgaattgcatattcgtgaatcatcgagtctttgaacgcagcttgcactctatggatcttctatagagtacgcttgcttcagtatcataaccaacccacacataaaatttattttatgtggtgatggacaagctcggttaaatttaattattataccgattgtctaaaatacagcctctttgtaattttcattaaattacgaactacctagccatcgtgcttttttggtccaaccaaaaaacatataatctaggggttctgctagccagcagatattttaatgatctttaactatgatctgaagtcaagtgggactacccgctgaacttaagcatatcata

SEQ ID NO: 2 - DNA, 20 bp, synthetic construct
  misc_feature 1..20: note = ITS4 primer
  source 1..20: mol_type = other DNA
tcctccgcttattgatatgc

SEQ ID NO: 3 - DNA, 22 bp, synthetic construct
  misc_feature 1..22: note = ITS5 primer
  source 1..22: mol_type = other DNA
ggaagtaaaagtcgtaacaagg